European Patent Specification EP 3 670 529 B1, published January 24, 2024. Title: Acylated oxyntomodulin analogues. Applicant: DONG-A ST CO., LTD. The sequence listing filed with the application follows.

SEQUENCE LISTING (53 sequences)

SEQ ID NO: 1 - protein, 37 aa, Homo sapiens
HSQGTFTSDYSKYLDSRRAQDFVQWLMNTKRNRNNIA

SEQ ID NO: 2 - protein, 30 aa, Artificial Sequence
  oxyntomodulin analogue
  MOD_RES (10): Xaa=modified Lys; Lys([(2-(2-(2-aminoethoxy)ethoxy)acetoyl)2]-[gamma glutamicacid]-[octadecanoyl])
HSQGTFTSDXSKYLDSRRAQDFVQWLMNTK

SEQ ID NO: 3 - protein, 30 aa, Artificial Sequence
  oxyntomodulin analogue
  MOD_RES (2): Xaa=aminoisobutyric acid
  MOD_RES (10): Xaa=modified Lys; Lys([(2-(2-(2-aminoethoxy)ethoxy)acetoyl)2]-[gamma glutamicacid]-[octadecanoyl])
HXQGTFTSDXSKYLDSRRAQDFVQWLMNTK

SEQ ID NO: 4 - protein, 30 aa, Artificial Sequence
  oxyntomodulin analogue
  MOD_RES (2): Xaa=aminoisobutyric acid
  MOD_RES (10): Xaa=modified Lys; Lys([(2-(2-(2-aminoethoxy)ethoxy)acetoyl)2]-[gamma glutamicacid]-[octadecanoyl])
  MOD_RES (16): Xaa=aminoisobutyric acid
HXQGTFTSDXSKYLDXRRAQDFVQWLMNTK

SEQ ID NO: 5 - protein, 30 aa, Artificial Sequence; identical to SEQ ID NO: 2
  oxyntomodulin analogue
  MOD_RES (10): Xaa=modified Lys; Lys([(2-(2-(2-aminoethoxy)ethoxy)acetoyl)2]-[gamma glutamicacid]-[octadecanoyl])
  MOD_RES (30): AMIDATION, C-terminal amidation

SEQ ID NO: 6 - protein, 37 aa, Artificial Sequence
  oxyntomodulin analogue
  MOD_RES (10): Xaa=modified Lys; Lys([(2-(2-(2-aminoethoxy)ethoxy)acetoyl)2]-[gamma glutamicacid]-[octadecanoyl])
HSQGTFTSDXSKYLDSRRAQDFVQWLMNTKRNRNNIA

SEQ ID NO: 7 - protein, 30 aa, Artificial Sequence; identical to SEQ ID NO: 4
  oxyntomodulin analogue
  MOD_RES (2): Xaa=aminoisobutyric acid
  MOD_RES (10): Xaa=modified Lys; Lys([(2-(2-(2-aminoethoxy)ethoxy)acetoyl)2]-[gamma glutamicacid]-[octadecanoyl])
  MOD_RES (16): Xaa=aminoisobutyric acid
  MOD_RES (30): AMIDATION, C-terminal amidation

SEQ ID NO: 8 - protein, 37 aa, Artificial Sequence
  oxyntomodulin analogue
  MOD_RES (2): Xaa=aminoisobutyric acid
  MOD_RES (10): Xaa=modified Lys; Lys([(2-(2-(2-aminoethoxy)ethoxy)acetoyl)2]-[gamma glutamicacid]-[octadecanoyl])
  MOD_RES (16): Xaa=aminoisobutyric acid
HXQGTFTSDXSKYLDXRRAQDFVQWLMNTKRNRNNIA

SEQ ID NO: 9 - protein, 30 aa, Artificial Sequence; identical to SEQ ID NO: 4
  oxyntomodulin analogue
  MOD_RES (2): Xaa=aminoisobutyric acid
  MOD_RES (10): Xaa=modified Lys; Lys([(2-(2-(2-aminoethoxy)ethoxy)acetoyl)2]-[gamma glutamicacid]-[icosanoyl])
  MOD_RES (16): Xaa=aminoisobutyric acid

SEQ ID NO: 10 - protein, 30 aa, Artificial Sequence; identical to SEQ ID NO: 4
  oxyntomodulin analogue
  MOD_RES (2): Xaa=aminoisobutyric acid
  MOD_RES (10): Xaa=modified Lys; Lys([(2-(2-(2-aminoethoxy)ethoxy)acetoyl)2]-[(gamma glutamicacid)2]-[octadecanoyl])
  MOD_RES (16): Xaa=aminoisobutyric acid

SEQ ID NO: 11 - protein, 30 aa, Artificial Sequence; identical to SEQ ID NO: 4
  oxyntomodulin analogue
  MOD_RES (2): Xaa=aminoisobutyric acid
  MOD_RES (10): Xaa=modified Lys; Lys([(2-(2-(2-aminoethoxy)ethoxy)acetoyl)3]-[gamma glutamicacid]-[octadecanoyl])
  MOD_RES (16): Xaa=aminoisobutyric acid

SEQ ID NO: 12 - protein, 30 aa, Artificial Sequence; identical to SEQ ID NO: 4
  oxyntomodulin analogue
  MOD_RES (2): Xaa=aminoisobutyric acid
  MOD_RES (10): Xaa=modified Lys; Lys([Gly-Gly-Ser-Gly-Ser-Gly]-[gamma glutamic acid]-[octadecanoyl])
  MOD_RES (16): Xaa=aminoisobutyric acid

SEQ ID NO: 13 - protein, 30 aa, Artificial Sequence
  oxyntomodulin analogue
  MOD_RES (2): Xaa=aminoisobutyric acid
  MOD_RES (10): Xaa=modified Lys; Lys([(2-(2-(2-aminoethoxy)ethoxy)acetoyl)2]-[gamma glutamicacid]-[octadecanoyl])
  MOD_RES (16): Xaa=aminoisobutyric acid
HXQGTFTSDXSKYLDXRRAQDFVQWLLRAK

SEQ ID NO: 14 - protein, 30 aa, Artificial Sequence; identical to SEQ ID NO: 4
  oxyntomodulin analogue
  MOD_RES (2): Xaa=aminoisobutyric acid
  MOD_RES (10): Xaa=modified Lys; Lys([(2-(2-(2-aminoethoxy)ethoxy)acetoyl)2]-[gamma glutamicacid]-[17-aminocarbonylheptadecanoyl])
  MOD_RES (16): Xaa=aminoisobutyric acid

SEQ ID NO: 15 - protein, 30 aa, Artificial Sequence
  oxyntomodulin analogue
  MOD_RES (2): Xaa=aminoisobutyric acid
  MOD_RES (10): Xaa=modified Lys; Lys([(2-(2-(2-aminoethoxy)ethoxy)acetoyl)2]-[gamma glutamicacid]-[octadecanoyl])
  MOD_RES (16)..(20): Lactam bridge bewteen the side chains at positions 16 and 20
HXQGTFTSDXSKYLDERRAKDFVQWLMNTK

SEQ ID NO: 16 - protein, 30 aa, Artificial Sequence
  oxyntomodulin analogue
  MOD_RES (2): Xaa=aminoisobutyric acid
  MOD_RES (16): Xaa=modified Lys; Lys([(2-(2-(2-aminoethoxy)ethoxy)acetoyl)2]-[gamma glutamicacid]-[octadecanoyl])
HXQGTFTSDYSKYLDXRRAQDFVQWLMNTK

SEQ ID NO: 17 - protein, 30 aa, Artificial Sequence
  oxyntomodulin analogue
  MOD_RES (2): Xaa=aminoisobutyric acid
  MOD_RES (16): Xaa=aminoisobutyric acid
  MOD_RES (20): Xaa=modified Lys; Lys([(2-(2-(2-aminoethoxy)ethoxy)acetoyl)2]-[gamma glutamicacid]-[octadecanoyl])
HXQGTFTSDYSKYLDXRRAXDFVQWLMNTK

SEQ ID NO: 18 - protein, 30 aa, Artificial Sequence; identical to SEQ ID NO: 4
  oxyntomodulin analogue
  MOD_RES (2): Xaa=aminoisobutyric acid
  MOD_RES (10): Xaa=modified Lys; Lys([(2-(2-(2-aminoethoxy)ethoxy)acetoyl)]-[gamma glutamic acid]-[octadecanoyl])
  MOD_RES (16): Xaa=aminoisobutyric acid

SEQ ID NO: 19 - protein, 30 aa, Artificial Sequence; identical to SEQ ID NO: 4
  oxyntomodulin analogue
  MOD_RES (2): Xaa=aminoisobutyric acid
  MOD_RES (10): Xaa=modified Lys; Lys([(2-(2-(2-aminoethoxy)ethoxy)acetoyl)4]-[gamma glutamicacid]-[octadecanoyl])
  MOD_RES (16): Xaa=aminoisobutyric acid

SEQ ID NO: 20 - protein, 30 aa, Artificial Sequence; identical to SEQ ID NO: 15
  oxyntomodulin analogue
  MOD_RES (2): Xaa=aminoisobutyric acid
  MOD_RES (10): Xaa=modified Lys; Lys([(2-(2-(2-aminoethoxy)ethoxy)acetoyl)2]-[gamma glutamicacid]-[octadecanoyl])
  MOD_RES (16)..(20): Lactam bridge bewteen the side chains at positions 16 and 20
  MOD_RES (30): AMIDATION, C-terminal amidation

SEQ ID NO: 21 - protein, 30 aa, Artificial Sequence; identical to SEQ ID NO: 15
  oxyntomodulin analogue
  MOD_RES (2): Xaa=aminoisobutyric acid
  MOD_RES (10): Xaa=modified Lys; Lys([(2-(2-(2-aminoethoxy)ethoxy)acetoyl)3]-[gamma glutamicacid]-[octadecanoyl])
  MOD_RES (16)..(20): Lactam bridge bewteen the side chains at positions 16 and 20

SEQ ID NO: 22 - protein, 30 aa, Artificial Sequence
  oxyntomodulin analogue
  MOD_RES (2): Xaa=aminoisobutyric acid
  MOD_RES (10): Xaa=modified Lys; Lys([(2-(2-(2-aminoethoxy)ethoxy)acetoyl)2]-[gamma glutamicacid]-[octadecanoyl])
  MOD_RES (16)..(20): Lactam bridge bewteen the side chains at positions 16 and 20
HXQGTFTSDXSKYLDKRRAEDFVQWLMNTK

SEQ ID NO: 23 - protein, 30 aa, Artificial Sequence
  oxyntomodulin analogue
  MOD_RES (2): Xaa=aminoisobutyric acid
  MOD_RES (10): Xaa=modified Lys; Lys([(2-(2-(2-aminoethoxy)ethoxy)acetoyl)2]-[gamma glutamicacid]-[octadecanoyl])
  MOD_RES (16)..(20): 1,3-phenylenedimethyl cross linking between 16 and 20
HXQGTFTSDXSKYLDCRRACDFVQWLMNTK

SEQ ID NO: 24 - protein, 30 aa, Artificial Sequence
  oxyntomodulin analogue
  MOD_RES (2): Xaa=aminoisobutyric acid
  MOD_RES (10): Xaa=modified Lys; Lys([(2-(2-(2-aminoethoxy)ethoxy)acetoyl)2]-[gamma glutamicacid]-[octadecanoyl])
  MOD_RES (16)..(20): 1,4-piperazinyl cross linking between 16 and 20
HXQGTFTSDXSKYLDERRAEDFVQWLMNTK

SEQ ID NO: 25 - protein, 30 aa, Artificial Sequence; identical to SEQ ID NO: 15
  oxyntomodulin analogue
  MOD_RES (2): Xaa=aminoisobutyric acid
  MOD_RES (10): Xaa=modified Lys; Lys([(2-(2-(2-aminoethoxy)ethoxy)acetoyl)4]-[gamma glutamicacid]-[octadecanoyl])
  MOD_RES (16)..(20): Lactam bridge bewteen the side chains at positions 16 and 20
  MOD_RES (30): AMIDATION, C-terminal amidation

SEQ ID NO: 26 - protein, 30 aa, Artificial Sequence; identical to SEQ ID NO: 15
  oxyntomodulin analogue
  MOD_RES (2): Xaa=aminoisobutyric acid
  MOD_RES (10): Xaa=modified Lys; Lys([(2-(2-(2-aminoethoxy)ethoxy)acetoyl)4]-[gamma glutamicacid]-[octadecanoyl])
  MOD_RES (16)..(20): Lactam bridge bewteen the side chains at positions 16 and 20

SEQ ID NO: 27 - protein, 30 aa, Artificial Sequence
  oxyntomodulin analogue
  MOD_RES (2): Xaa=aminoisobutyric acid
  MOD_RES (10): Xaa=modified Lys; Lys([(2-(2-(2-aminoethoxy)ethoxy)acetoyl)2]-[gamma glutamicacid]-[octadecanoyl])
  MOD_RES (16)..(20): Lactam bridge bewteen the side chains at positions 16 and 20
HXQGTFTSDXSKYLDDRRAKDFVQWLMNTK

SEQ ID NO: 28 - protein, 30 aa, Artificial Sequence
  oxyntomodulin analogue
  MOD_RES (2): Xaa=aminoisobutyric acid
  MOD_RES (10): Xaa=modified Lys; Lys([(2-(2-(2-aminoethoxy)ethoxy)acetoyl)2]-[gamma glutamicacid]-[octadecanoyl])
  MOD_RES (16)..(20): Lactam bridge bewteen the side chains at positions 16 and 20
HXQGTFTSDXSKYLDKRRADDFVQWLMNTK

SEQ ID NO: 29 - protein, 30 aa, Artificial Sequence; identical to SEQ ID NO: 23
  oxyntomodulin analogue
  MOD_RES (2): Xaa=aminoisobutyric acid
  MOD_RES (10): Xaa=modified Lys; Lys([(2-(2-(2-aminoethoxy)ethoxy)acetoyl)2]-[gamma glutamicacid]-[octadecanoyl])
  MOD_RES (16)..(20): di-sulfide bridge bewteen the side chains at positions 16 and 20

SEQ ID NO: 30 - protein, 30 aa, Artificial Sequence; identical to SEQ ID NO: 24
  oxyntomodulin analogue
  MOD_RES (2): Xaa=aminoisobutyric acid
  MOD_RES (10): Xaa=modified Lys; Lys([(2-(2-(2-aminoethoxy)ethoxy)acetoyl)2]-[gamma glutamicacid]-[octadecanoyl])
  MOD_RES (16)..(20): 1,4-phenylenediamino cross linking between 16 and 20

SEQ ID NO: 31 - protein, 30 aa, Artificial Sequence; identical to SEQ ID NO: 24
  oxyntomodulin analogue
  MOD_RES (2): Xaa=aminoisobutyric acid
  MOD_RES (10): Xaa=modified Lys; Lys([(2-(2-(2-aminoethoxy)ethoxy)acetoyl)2]-[gamma glutamicacid]-[octadecanoyl])
  MOD_RES (16)..(20): 1,2-ethylenediamino cross linking between 16 and 20

SEQ ID NO: 32 - protein, 30 aa, Artificial Sequence
  oxyntomodulin analogue
  MOD_RES (2): Xaa=aminoisobutyric acid
  MOD_RES (10): Xaa=modified Lys; Lys([(2-(2-(2-aminoethoxy)ethoxy)acetoyl)2]-[gamma glutamicacid]-[octadecanoyl])
  MOD_RES (16)..(20): 1,4-phenylenebiscarbonyl cross linking between 16 and 20
HXQGTFTSDXSKYLDKRRAKDFVQWLMNTK

SEQ ID NO: 33 - protein, 30 aa, Artificial Sequence; identical to SEQ ID NO: 22
  oxyntomodulin analogue
  MOD_RES (2): Xaa=aminoisobutyric acid
  MOD_RES (10): Xaa=modified Lys; Lys([(2-(2-(2-aminoethoxy)ethoxy)acetoyl)2]-[gamma glutamicacid]-[octadecanoyl])
  MOD_RES (16)..(20): 4-carbonylpiperidin-1-yl cross linking between 16 and 20

SEQ ID NO: 34 - protein, 30 aa, Artificial Sequence; identical to SEQ ID NO: 15
  oxyntomodulin analogue
  MOD_RES (2): Xaa=aminoisobutyric acid
  MOD_RES (10): Xaa=modified Lys; Lys([(2-(2-(2-aminoethoxy)ethoxy)acetoyl)2]-[gamma glutamicacid]-[octadecanoyl])
  MOD_RES (16)..(20): 1-aminocyclohexan-4-carbonyl cross linking between 16 and 20

SEQ ID NO: 35 - protein, 30 aa, Artificial Sequence; identical to SEQ ID NO: 15
  oxyntomodulin analogue
  MOD_RES (2): Xaa=aminoisobutyric acid
  MOD_RES (10): Xaa=modified Lys; Lys([(2-(2-(2-aminoethoxy)ethoxy)acetoyl)2]-[gamma glutamicacid]-[octadecanoyl])
  MOD_RES (16)..(20): 4-aminobenzoyl cross linking between 16 and 20

SEQ ID NO: 36 - protein, 30 aa, Artificial Sequence; identical to SEQ ID NO: 15
  oxyntomodulin analogue
  MOD_RES (2): Xaa=aminoisobutyric acid
  MOD_RES (10): Xaa=modified Lys; Lys([(2-(2-(2-aminoethoxy)ethoxy)acetoyl)2]-[gamma glutamicacid]-[octadecanoyl])
  MOD_RES (16)..(20): glycine cross linking between 16 and 20

SEQ ID NO: 37 - protein, 30 aa, Artificial Sequence; identical to SEQ ID NO: 15
  oxyntomodulin analogue
  MOD_RES (2): Xaa=aminoisobutyric acid
  MOD_RES (10): Xaa=modified Lys; Lys([(2-(2-(2-aminoethoxy)ethoxy)acetoyl)2]-[gamma glutamicacid]-[octadecanoyl])
  MOD_RES (16)..(20): leucine cross linking between 16 and 20

SEQ ID NO: 38 - protein, 30 aa, Artificial Sequence; identical to SEQ ID NO: 27
  oxyntomodulin analogue
  MOD_RES (2): Xaa=aminoisobutyric acid
  MOD_RES (10): Xaa=modified Lys; Lys([(2-(2-(2-aminoethoxy)ethoxy)acetoyl)2]-[gamma glutamicacid]-[octadecanoyl])
  MOD_RES (16)..(20): glycine cross linking between 16 and 20

SEQ ID NO: 39 - protein, 30 aa, Artificial Sequence; identical to SEQ ID NO: 27
  oxyntomodulin analogue
  MOD_RES (2): Xaa=aminoisobutyric acid
  MOD_RES (10): Xaa=modified Lys; Lys([(2-(2-(2-aminoethoxy)ethoxy)acetoyl)2]-[gamma glutamicacid]-[octadecanoyl])
  MOD_RES (16)..(20): leucine cross linking between 16 and 20

SEQ ID NO: 40 - protein, 30 aa, Artificial Sequence
  oxyntomodulin analogue
  MOD_RES (2): Xaa=aminoisobutyric acid
  MOD_RES (16): Xaa=aminoisobutyric acid
HXQGTFTSDKSKYLDXRRAQDFVQWLMNTK

SEQ ID NO: 41 - protein, 30 aa, Artificial Sequence
  oxyntomodulin analogue
  MOD_RES (2): Xaa=aminoisobutyric acid
  MOD_RES (9): aa=modified Lys; Lys([(2-(2-(2-aminoethoxy)ethoxy)acetoyl)2]-[gammaglutamicacid]-[ octadecanoyl])
  MOD_RES (16): Xaa=aminoisobutyric acid
HXQGTFTSXYSKYLDXRRAQDFVQWLMNTK

SEQ ID NO: 42 - protein, 30 aa, Artificial Sequence
  oxyntomodulin analogue
  MOD_RES (30): Xaa=modified Lys; Lys([(2-(2-(2-aminoethoxy)ethoxy)acetoyl)2]-[gammaglutamicacid]-[ octadecanoyl])
HSQGTFTSDYSKYLDSRRAQDFVQWLMNTX

SEQ ID NO: 43 - protein, 30 aa, Artificial Sequence; identical to SEQ ID NO: 4
  oxyntomodulin analogue
  MOD_RES (2): Xaa=aminoisobutyric acid
  MOD_RES (10): Xaa=modified Lys; Lys([(2-(2-(2-aminoethoxy)ethoxy)acetoyl)2]-[gammaglutamicacid]-[ 15-carboxypentadecanoyl])
  MOD_RES (16): Xaa=aminoisobutyric acid

SEQ ID NO: 44 - protein, 30 aa, Artificial Sequence; identical to SEQ ID NO: 4
  oxyntomodulin analogue
  MOD_RES (2): Xaa=aminoisobutyric acid
  MOD_RES (10): Xaa=modified Lys; Lys([(2-(2-(2-aminoethoxy)ethoxy)acetoyl)2]-[gammaglutamicacid]-[ 17-carboxyheptadecanoyl])
  MOD_RES (16): Xaa=aminoisobutyric acid

SEQ ID NO: 45 - protein, 30 aa, Artificial Sequence; identical to SEQ ID NO: 4
  oxyntomodulin analogue
  MOD_RES (2): Xaa=aminoisobutyric acid
  MOD_RES (10): Xaa=modified Lys; Lys([(2-(2-(2-aminoethoxy)ethoxy)acetoyl)2]-[gammaglutamicacid]-[ 19-carboxynonadecanoyl])
  MOD_RES (16): Xaa=aminoisobutyric acid

SEQ ID NO: 46 - protein, 30 aa, Artificial Sequence; identical to SEQ ID NO: 4
  oxyntomodulin analogue
  MOD_RES (2): Xaa=aminoisobutyric acid
  MOD_RES (10): Xaa=modified Lys; Lys([(2-(2-(2-aminoethoxy)ethoxy)acetoyl)2]-[gammaglutamicacid]-[ 15-(N-(carboxymethyl)amino)carbonylpentadecanoyl])
  MOD_RES (16): Xaa=aminoisobutyric acid

SEQ ID NO: 47 - protein, 30 aa, Artificial Sequence; identical to SEQ ID NO: 4
  oxyntomodulin analogue
  MOD_RES (2): Xaa=aminoisobutyric acid
  MOD_RES (10): Xaa=modified Lys; Lys([(2-(2-(2-aminoethoxy)ethoxy)acetoyl)2]-[gammaglutamicacid]-[ 15-(N-(1S)-(1-carboxy-2-methylpropyl)amino)carbonylpentadecanoyl] )
  MOD_RES (16): Xaa=aminoisobutyric acid

SEQ ID NO: 48 - protein, 31 aa, Artificial Sequence
  oxyntomodulin analogue
  MOD_RES (2): Xaa=aminoisobutyric acid
  MOD_RES (16)..(20): Lactam bridge bewteen the side chains at positions 16 and 20
HXQGTFTSDYSKYLDEKRAKEFVQWLMNTKC

SEQ ID NO: 49 - protein, 32 aa, Artificial Sequence
  oxyntomodulin analogue
  VARIANT (2): Xaa=Ser or aminoisobutyric acid
  VARIANT (9): Xaa=Asp or modified Lys
  VARIANT (10): Xaa=Tyr or modified Lys
  VARIANT (11): Xaa=Ser or modified Lys
  VARIANT (12): Xaa=Lys or modified Lys
  VARIANT (13): Xaa=Tyr or modified Lys
  VARIANT (14): Xaa=Leu or modified Lys
  VARIANT (15): Xaa=Asp or modified Lys
  VARIANT (16): Xaa=Ser, aminoisobutyric acid or modified Lys
  VARIANT (20): Xaa=Gln or modified Lys
  VARIANT (27): Xaa=Met or Leu
  VARIANT (28): Xaa=Asn or Arg
  VARIANT (29): Xaa=Thr or Ala
  VARIANT (30): Xaa=Lys or modified Lys
  VARIANT (31): Xaa=optional, but when present is RNRNNIA(ArgAsnArgAsnAsnIleAla)
  VARIANT (32): Xaa=optional, when 31 is RNRNNIA(ArgAsnArgAsnAsnIleAla), Xaa is doesn't exist or is modified Lys
HXQGTFTSXXXXXXXXRRAXDFVQWLXXXXXX

SEQ ID NO: 50 - protein, 32 aa, Artificial Sequence
  oxyntomodulin analogue
  VARIANT (2): Xaa=Ser or aminoisobutyric acid
  VARIANT (10): Xaa=Tyr or modified Lys
  VARIANT (16): Xaa=Ser, aminoisobutyric acid or modified Lys
  VARIANT (20): Xaa=Gln or modified Lys
  VARIANT (27): Xaa=Met or Leu
  VARIANT (28): Xaa=Asn or Arg
  VARIANT (29): Xaa=Thr or Ala
  VARIANT (30): Xaa=Lys or modified Lys
  VARIANT (31): Xaa=optional, but when present is RNRNNIA(ArgAsnArgAsnAsnIleAla)
  VARIANT (32): Xaa=optional, when 31 is RNRNNIA(ArgAsnArgAsnAsnIleAla), Xaa is doesn't exist or is modified Lys
HXQGTFTSDXSKYLDXRRAXDFVQWLXXXXXX

SEQ ID NO: 51 - protein, 7 aa, Artificial Sequence
  oxyntomodulin peptide
RNRNNIA

SEQ ID NO: 52 - protein, 6 aa, Artificial Sequence
  artificial sequence
GGSGSG

SEQ ID NO: 53 - protein, 30 aa, Artificial Sequence
  oxyntomodulin analogue
  VARIANT (2): Xaa=Ser or aminoisobutyric acid
  VARIANT (10): Xaa=modified Lys
  VARIANT (16): Xaa=Asp, Glu, Cys, Hcy (Homocysteine), Lys or Orn (Ornithine)
  VARIANT (20): Xaa=Asp, Glu, Cys, Hcy (Homocysteine), Lys or Orn (Ornithine)
HXQGTFTSDXSKYLDXRRAXDFVQWLMNTK